European Patent Specification EP 3 746 064 B1, published April 16, 2025. Title: Compounds for the treatment of acute brain injury. Applicant: Copenhagen University. The sequence listing filed with the application follows.

SEQUENCE LISTING (12 sequences)

SEQ ID NO: 1 - DNA, 19 bp, Artificial Sequence
  CD14 (F)
aatctaccgaccatggagc

SEQ ID NO: 2 - DNA, 19 bp, Artificial Sequence
  CD14 (R)
actttcctcgtctagctcg

SEQ ID NO: 3 - DNA, 20 bp, Artificial Sequence
  IL-6 (F)
ctctgggaaatcgtggaaat

SEQ ID NO: 4 - DNA, 20 bp, Artificial Sequence
  IL-6 (R)
ccagtttggtagcatccatc

SEQ ID NO: 5 - DNA, 21 bp, Artificial Sequence
  MMP9 (F)
cagccgacttttgtggtcttc

SEQ ID NO: 6 - DNA, 20 bp, Artificial Sequence
  MMP9 (R)
cggccgtagagactgcttct

SEQ ID NO: 7 - DNA, 19 bp, Artificial Sequence
  GFAP (F)
ggagatgcgggatggtgag

SEQ ID NO: 8 - DNA, 20 bp, Artificial Sequence
  GFAP (R)
accacgtccttgtgctcctg

SEQ ID NO: 9 - DNA, 20 bp, Artificial Sequence
  Rpl13a (F)
ggaggggcaggttctggtat

SEQ ID NO: 10 - DNA, 20 bp, Artificial Sequence
  Rpl13a (R)
tgttgatgccttcacagcgt

SEQ ID NO: 11 - DNA, 20 bp, Artificial Sequence
  SDHA (F)
gcccatgccagggaagatta

SEQ ID NO: 12 - DNA, 20 bp, Artificial Sequence
  SDHA (R)
tgttccccaaacggcttctt